European Patent Specification EP 3 538 667 B1, published March 20, 2024. Title: METHODS OF PERFORMING NUCLEIC ACID STABILIZATION AND SEPARATION. Applicant: Qvella Corporation. The sequence listing filed with the application follows.

SEQUENCE LISTING (4 sequences)

SEQ ID NO: 1 - DNA, 20 bp, Artificial
  LAMP1 forward primer
accgtcctgctcttccagtt

SEQ ID NO: 2 - DNA, 18 bp, Artificial
  LAMP1 reverse primer
ggcagggtctctggcgtc

SEQ ID NO: 3 - DNA, 19 bp, Artificial
  GAPDH forward primer
gccacatcgctcagacacc

SEQ ID NO: 4 - DNA, 22 bp, Artificial
  GAPDH reverse primer
gttaaaagcagccctggtgacc